European Patent Application EP 4 257 617 A1, published October 11, 2023. Title: ANTIGEN-BINDING PROTEIN TARGETING CD70 AND USE THEREOF. Applicant: CURE GENETICS CO., LTD. Application EP21899983.7. The sequence listing filed with the application follows.

SEQUENCE LISTING (94 sequences)

SEQ ID NO: 1 - protein, 8 aa, Artificial Sequence
  1C HCDR1; H3 HCDR1; 1H HCDR1
GKPFSFYF

SEQ ID NO: 2 - protein, 7 aa, Artificial Sequence
  1C HCDR2; H3 HCDR2; 1H HCDR2
ITGDGMT

SEQ ID NO: 3 - protein, 13 aa, Artificial Sequence
  1C HCDR3
YADAWAGAGREEY

SEQ ID NO: 4 - protein, 13 aa, Artificial Sequence
  H3 HCDR3
YADAWAGAVRAEY

SEQ ID NO: 5 - protein, 13 aa, Artificial Sequence
  1H HCDR3
YADVWAGAGRDEY

SEQ ID NO: 6 - protein, 8 aa, Artificial Sequence
  1F HCDR1
GKRFSFYF

SEQ ID NO: 7 - protein, 7 aa, Artificial Sequence
  1F HCDR2; 5H HCDR2
ITGDGRT

SEQ ID NO: 8 - protein, 13 aa, Artificial Sequence
  1F HCDR3
YADAFAGAGRDEY

SEQ ID NO: 9 - protein, 8 aa, Artificial Sequence
  5H HCDR1
GKIFSFYF

SEQ ID NO: 10 - protein, 13 aa, Artificial Sequence
  5H HCDR3
YADVFARAGRDEY

SEQ ID NO: 11 - protein, 8 aa, Artificial Sequence
  3H HCDR1
GNILRFNA

SEQ ID NO: 12 - protein, 8 aa, Artificial Sequence
  3H HCDR2
MAGARTNY

SEQ ID NO: 13 - protein, 10 aa, Artificial Sequence
  3H HCDR3
DRVYGPPYEY

SEQ ID NO: 14 - protein, 8 aa, Artificial Sequence
  1G HCDR1
SGIIFNSD

SEQ ID NO: 15 - protein, 7 aa, Artificial Sequence
  1G HCDR2
LTSNMRT

SEQ ID NO: 16 - protein, 13 aa, Artificial Sequence
  1G HCDR3
NVNRMTSYGPRDY

SEQ ID NO: 17 - protein, 8 aa, Artificial Sequence
  L1 HCDR1
GRTFSSYA

SEQ ID NO: 18 - protein, 8 aa, Artificial Sequence
  L1 HCDR2
INWSDGST

SEQ ID NO: 19 - protein, 17 aa, Artificial Sequence
  L1 HCDR3
AAGCCGVADAPLNALDA

SEQ ID NO: 20 - protein, 8 aa, Artificial Sequence
  5A HCDR1
ESIFNNYV

SEQ ID NO: 21 - protein, 7 aa, Artificial Sequence
  5A HCDR2
ISTDGSA

SEQ ID NO: 22 - protein, 6 aa, Artificial Sequence
  5A HCDR3
TAGLQY

SEQ ID NO: 23 - protein, 8 aa, Artificial Sequence
  7D HCDR1; 5B HCDR1
GFTFDDYA

SEQ ID NO: 24 - protein, 8 aa, Artificial Sequence
  7D HCDR2
IRRSDGST

SEQ ID NO: 25 - protein, 18 aa, Artificial Sequence
  7D HCDR3
AVDRYGQSWHEGRGALDA

SEQ ID NO: 26 - protein, 8 aa, Artificial Sequence
  L2 HCDR1
GFTVDDYV

SEQ ID NO: 27 - protein, 8 aa, Artificial Sequence
  L2 HCDR2
ISSNDGST

SEQ ID NO: 28 - protein, 18 aa, Artificial Sequence
  L2 HCDR3
AAKYAPYGLEYWEGGMDY

SEQ ID NO: 29 - protein, 8 aa, Artificial Sequence
  1E HCDR1
GFAFDDYA

SEQ ID NO: 30 - protein, 8 aa, Artificial Sequence
  1E HCDR2
MSSSDGST

SEQ ID NO: 31 - protein, 18 aa, Artificial Sequence
  1E HCDR3
AAGVNYYREDGCPGALDY

SEQ ID NO: 32 - protein, 8 aa, Artificial Sequence
  5B HCDR2
FRSSDGNI

SEQ ID NO: 33 - protein, 19 aa, Artificial Sequence
  5B HCDR3
AAYSVLLRPWVLCEGSYDY

SEQ ID NO: 34 - protein, 119 aa, Artificial Sequence
  CD70-sdAb-1C
EVQVVESGGGMVQAGRSLRLSCAASGKPFSFYFMGWYRQAPGNQRELVALITGDGMTNYADSVEGRFTISRDNAKNTMYLEMNSLKPEDTAVYYCYADAWAGAGREEYWGQGTQVSVSS

SEQ ID NO: 35 - protein, 125 aa, Artificial Sequence
  CD70-sdAb-1E
EVQVVESGGGLVQAGGSLRLSCAASGFAFDDYAIGWFRQAPGKEQERVSCMSSSDGSTYYADSVKGRFTISSDNAKNTVYLQMNSLKPEDTAVYYCAAGVNYYREDGCPGALDYWGQGTQVTVSS

SEQ ID NO: 36 - protein, 119 aa, Artificial Sequence
  CD70-sdAb-1F
EVQVVESGGGMVQAGGSLRLSCAASGKRFSFYFMGWYRQAPGKQRELVALITGDGRTNYAGSVEGRFTISRDNAKNTLYLQMNSMKPEDTAVYYCYADAFAGAGRDEYWGQGTQVSVSS

SEQ ID NO: 37 - protein, 118 aa, Artificial Sequence
  CD70-sdAb-1G
QLQLVESGGGLVQLGGSLTLSCTASGIIFNSDYVGWYRQAPGSDRELVALTSNMRTNYADSVEGRFTISRDNAKNTVYLQMNSLKPEDTAVYYCNVNRMTSYGPRDYWGQGTQVTVSS

SEQ ID NO: 38 - protein, 119 aa, Artificial Sequence
  CD70-sdAb-1H
EVQLVESGGGMVQAGGSLRLSCAASGKPFSFYFMGWYRQAPGKQRELVALITGDGMTNYADSVEGRFTISRDNAKNTMYLQMNSLKPEDTAVYYCYADVWAGAGRDEYWGQGTRVTVSS

SEQ ID NO: 39 - protein, 117 aa, Artificial Sequence
  CD70-sdAb-3H
QLQLVESGGGLVQPGGSLRLSCAASGNILRFNAVGWYRQAPGKQRDLVAAMAGARTNYADSVEGRFTISGNNANNTVYLQMNSLKPEDTGVYYCGADRVYGPPYEYGGRGTQVTVLS

SEQ ID NO: 40 - protein, 112 aa, Artificial Sequence
  CD70-sdAb-5A
EVQLVESGGGLVQAGGSLRLSCAASESIFNNYVMAWYRQPPGKQREAVAQISTDGSAYYQDRVKGRFTISRDNAKNLVNLQMSSLKPEDTAVYYCTAGLQYWGQGTQVTVSS

SEQ ID NO: 41 - protein, 126 aa, Artificial Sequence
  CD70-sdAb-5B
QVQLVESGGGLVQAGGSLRLSCAASGFTFDDYAIGWFRQAPGKEPEGVSCFRSSDGNIYYSDSVRGRFTISSDNAKNTVYLQMNRLKPEDTAVYYCAAYSVLLRPWVLCEGSYDYWGQGTQVTVSS

SEQ ID NO: 42 - protein, 119 aa, Artificial Sequence
  CD70-sdAb-5H
EVQLVESGGGMVQAGGSLRLSCAAPGKIFSFYFMGWYRQAPGKQRELVALITGDGRTNYADSVEGRFTISRDNAKNTVYLQMNSLKPEDTAVYYCYADVFARAGRDEYWGQGTQVSVSS

SEQ ID NO: 43 - protein, 125 aa, Artificial Sequence
  CD70-sdAb-7D
EVQLVESGGGLVQAGGSLRLSCAASGFTFDDYAIGWFRQAPGKEQEGVSCIRRSDGSTWYANSVKGRFTISNDNAKNTVYLQMNSLKPEDTAVYYCAVDRYGQSWHEGRGALDAWGQGTLVTVSS

SEQ ID NO: 44 - protein, 119 aa, Artificial Sequence
  CD70-sdAb-H3
QVQLVESGGGMVQAGRSLRLSCAASGKPFSFYFMGWYRQAPGKERELVALITGDGMTNYADSVEGRFTISRDNAKNTLYLEMNSLKPEDTAVYYCYADAWAGAVRAEYWGQGTQVSVSS

SEQ ID NO: 45 - protein, 125 aa, Artificial Sequence
  CD70-sdAb-L2
EVQLVESGGGLVQAGGSLRLSCAASGFTVDDYVIGWFRQAPGKEHEGVSCISSNDGSTWYADSVKGRFTISSDNAKNTMYLQMNSLKPEDTAVYYCAAKYAPYGLEYWEGGMDYWGKGTLVTVSS

SEQ ID NO: 46 - protein, 124 aa, Artificial Sequence
  CD70-sdAb-L1
EVQVVESGGGLVQAGGSLRLSCAASGRTFSSYAMGWVRQAPGKDQEFVAAINWSDGSTYYADSVKGRFTIARDNAKNTAFLQMNSLKPEDTAVYYCAAGCCGVADAPLNALDAWGQGTLVTVSS

SEQ ID NO: 47 - DNA, 357 bp, Artificial Sequence
  Nucleic acid sequence of CD70-sdAb-1C
gaggtgcaggtggtggagtcggggggaggaatggtgcaggctgggcgatctctgagactctcctgtgctgcctctggaaagcccttcagtttctatttcatgggatggtatcgccaggctccaggaaaccagcgcgagttggtcgcccttattaccggtgatggtatgacaaactatgcagactccgtggagggccgattcaccatctccagagacaacgccaagaatacaatgtatctcgaaatgaacagcctgaaacctgaggacacagccgtctattattgctatgcagatgcttgggcgggggccggccgcgaagagtactggggccaggggacccaggtcagcgtctcctca

SEQ ID NO: 48 - DNA, 375 bp, Artificial Sequence
  Nucleic acid sequence of CD70-sdAb-1E
gaggtgcaggtggtggagtctgggggaggcttggtgcaggctggggggtctctgagactctcctgtgcagcctctggattcgctttcgatgattatgccataggctggttccgccaggccccagggaaggagcaggaaagagtctcatgtatgagtagtagtgatggtagcacatactatgcagactccgtgaagggccgattcaccatctccagtgacaacgccaagaacacggtgtatctgcaaatgaacagcctgaaacctgaggacacggccgtttattactgtgccgcaggggtcaattactatcgcgaggatgggtgcccgggcgcgttggactactggggccaggggacccaggtcaccgtctcctca

SEQ ID NO: 49 - DNA, 357 bp, Artificial Sequence
  Nucleic acid sequence of CD70-sdAb-1F
gaggtgcaggtggtggagtcggggggaggaatggtgcaggctgggggatctctgaggctctcctgtgcagcctctggaaagcgcttcagtttctattttatgggatggtaccgccaggctccaggaaagcagcgcgagttggtcgcccttattactggtgatggcaggacaaactatgcagggtccgtggagggccgattcaccatctccagagacaacgccaagaacacgctatatctgcaaatgaacagcatgaaacctgaggacacagccgtctattattgctatgcagatgcattcgcgggggccggccgcgatgagtactggggccaggggacccaggtcagcgtctcctca

SEQ ID NO: 50 - DNA, 354 bp, Artificial Sequence
  Nucleic acid sequence of CD70-sdAb-1G
cagttgcagctcgtggagtccgggggaggcttggtgcaacttggggggtctctgacgctctcctgtacagcctctgggattatcttcaatagcgattacgtgggctggtaccgccaggctccagggtcggatcgcgagttggtcgcacttactagtaatatgaggacaaactatgcagactccgtggagggccgattcaccatctccagagacaacgccaagaatacggtgtatctgcaaatgaacagcctgaaacctgaggacacggccgtctattattgtaatgtaaatagaatgacctcctatgggcctcgggactactggggccaggggacccaggtcaccgtctcctcc

SEQ ID NO: 51 - DNA, 357 bp, Artificial Sequence
  Nucleic acid sequence of CD70-sdAb-1H
gaggtgcagctggtggagtctggtggaggaatggtgcaggctgggggatctctgagactctcctgtgctgcctctggaaagcccttcagtttctatttcatgggatggtaccgccaggctccaggaaagcagcgcgagttggtcgcccttattaccggtgatggtatgacaaactatgcagactccgtggagggccgattcaccatctccagagacaacgccaagaacacaatgtatctgcaaatgaacagcctgaaacctgaggacacagccgtctattattgctatgcagatgtatgggcgggggccggccgcgatgagtactggggccaggggacccgggtcaccgtctcctca

SEQ ID NO: 52 - DNA, 351 bp, Artificial Sequence
  Nucleic acid sequence of CD70-sdAb-3H
cagttgcagctcgtggagtcgggtggaggcttggtgcagcctggggggtctctgagactctcctgtgcagcctctggaaacatcctcagattcaatgccgtgggctggtaccgccaggctccagggaagcagcgcgacttggtcgcggctatggctggtgcacggacaaactatgcagactccgtggagggccgattcaccatctccggaaacaacgccaacaacacggtttatctgcaaatgaacagcctgaaacctgaagacacaggcgtctactactgtggtgctgaccgcgtatatggtccgccgtatgaatatgggggccgggggacccaggtcaccgtcttgtca

SEQ ID NO: 53 - DNA, 336 bp, Artificial Sequence
  Nucleic acid sequence of CD70-sdAb-5A
gaggtgcagctggtggagtcggggggaggcttggtgcaggctggggggtctctgaggctctcctgtgcagcctctgaaagcatcttcaataattatgtcatggcctggtaccgccagcctccagggaagcagcgcgaggcggtcgcacaaattagtactgatggtagtgcgtactatcaggaccgagtgaagggccgattcactatctccagagacaacgccaagaacttggtgaatctgcaaatgagcagcctgaaacctgaggacacagccgtctattactgtactgcaggtctccagtactggggccaggggacccaggtcaccgtctcctca

SEQ ID NO: 54 - DNA, 378 bp, Artificial Sequence
  Nucleic acid sequence of CD70-sdAb-5B
caggtgcagctcgtggagtctggaggaggcttggtgcaggctggggggtctctgagactctcctgtgcagcctctggattcactttcgatgattatgccataggctggttccgccaggccccagggaaggagcctgagggggtctcatgtttcaggagtagtgatggtaacatatactattcagactccgtgaggggccgattcaccatctccagtgacaacgccaagaacacggtgtatctgcaaatgaacagactgaaacctgaggacacggccgtttactactgtgcagcctatagcgtactgctcaggccctgggtgttatgtgaaggctcatatgactactggggccaggggacccaggtcaccgtctcctca

SEQ ID NO: 55 - DNA, 357 bp, Artificial Sequence
  Nucleic acid sequence of CD70-sdAb-5H
gaggtgcagctggtggagtcagggggaggtatggtgcaggctgggggatctctgagactctcctgtgcagcccctggaaagatcttcagtttctatttcatgggatggtaccgccaggctccaggaaagcagcgcgagttggtcgcccttattaccggtgatggtaggacaaactatgcagactccgtggagggccgattcaccatctccagagacaacgccaagaacacggtgtatctgcaaatgaacagcctgaaacctgaggacacagccgtctattattgctatgcagatgtatttgcgagggccggccgcgatgagtactggggccaggggacccaggtcagcgtctcctca

SEQ ID NO: 56 - DNA, 375 bp, Artificial Sequence
  Nucleic acid sequence of CD70-sdAb-7D
gaggtgcagctggtggagtctgggggaggcttggtgcaggctggggggtctctgagactctcctgtgcagcctctggattcactttcgatgattatgccataggctggttccgccaggccccagggaaggagcaagagggggtctcatgtattagacgtagtgatggtagcacatggtatgcaaactccgtgaagggccgattcaccatctccaatgacaacgccaagaacacggtgtatctgcaaatgaacagcctgaaacctgaggacacggccgtttattactgcgcagtagatcgttacggtcagagttggcacgagggccgcggcgctttggacgcatggggccaggggaccctggtcactgtctcctca

SEQ ID NO: 57 - DNA, 357 bp, Artificial Sequence
  Nucleic acid sequence of CD70-sdAb-H3
caggtgcagctcgtggagtctgggggaggaatggtgcaggctgggcgatctctgagactctcctgtgctgcctctggaaagcccttcagtttctatttcatgggatggtatcgccaggctccaggaaaggagcgcgagttggtcgcccttattaccggtgatggtatgacaaactatgcagactccgtggagggccgattcaccatctccagagacaacgccaagaatacattgtatctcgaaatgaacagcctgaaacctgaggacacagccgtctattattgctatgcagatgcttgggcgggggccgttcgcgccgagtactggggccaggggacccaggtcagcgtctcctca

SEQ ID NO: 58 - DNA, 375 bp, Artificial Sequence
  Nucleic acid sequence of CD70-sdAb-L2
gaggtgcagctggtggagtccgggggaggcttggtgcaggctggggggtctctgagactctcctgtgcagcctctggattcactgtcgatgattatgtcataggctggttccgccaggccccagggaaggagcatgagggggtctcatgtattagtagtaatgatggtagtacatggtatgcagactccgtgaagggccgattcaccatctccagtgacaacgccaagaacacgatgtatctgcaaatgaacagcctgaaacctgaggacacggccgtttattactgtgcagctaaatacgcaccctacgggttggagtactgggagggaggcatggactactggggcaaagggaccctggtcaccgtctcctca

SEQ ID NO: 59 - DNA, 372 bp, Artificial Sequence
  Nucleic acid sequence of CD70-sdAb-L1
gaggtgcaggtggtggagtctgggggaggattggtgcaggctgggggctctctgagactctcctgtgcagcctctggacgcaccttcagttcatatgccatgggctgggtccgccaggctccagggaaggaccaagagtttgtagcggctattaactggagtgatggtagcacatactatgcagactccgtgaagggccgattcaccatcgccagagacaacgccaagaacacggcgtttctgcaaatgaacagcctgaaacctgaggacacggccgtgtattactgtgcagcagggtgttgcggagtagctgatgcccccctcaatgctttggacgcatggggccaggggaccctggtcactgtctcctca

SEQ ID NO: 60 - protein, 363 aa, Artificial Sequence
  CD70-CAR-1C
MALPVTALLLPLALLLHAARPEVQVVESGGGMVQAGRSLRLSCAASGKPFSFYFMGWYRQAPGNQRELVALITGDGMTNYADSVEGRFTISRDNAKNTMYLEMNSLKPEDTAVYYCYADAWAGAGREEYWGQGTQVSVSSTTTPAPRPPTPAPTIASQPLSLRPEACRPAAGGAVHTRGLDFACDIYIWAPLAGTCGVLLLSLVITLYCKRGRKKLLYIFKQPFMRPVQTTQEEDGCSCRFPEEEEGGCELRVKFSRSADAPAYKQGQNQLYNELNLGRREEYDVLDKRRGRDPEMGGKPRRKNPQEGLYNELQKDKMAEAYSEIGMKGERRRGKGHDGLYQGLSTATKDTYDALHMQALPPR

SEQ ID NO: 61 - protein, 369 aa, Artificial Sequence
  CD70-CAR-1E
MALPVTALLLPLALLLHAARPEVQVVESGGGLVQAGGSLRLSCAASGFAFDDYAIGWFRQAPGKEQERVSCMSSSDGSTYYADSVKGRFTISSDNAKNTVYLQMNSLKPEDTAVYYCAAGVNYYREDGCPGALDYWGQGTQVTVSSTTTPAPRPPTPAPTIASQPLSLRPEACRPAAGGAVHTRGLDFACDIYIWAPLAGTCGVLLLSLVITLYCKRGRKKLLYIFKQPFMRPVQTTQEEDGCSCRFPEEEEGGCELRVKFSRSADAPAYKQGQNQLYNELNLGRREEYDVLDKRRGRDPEMGGKPRRKNPQEGLYNELQKDKMAEAYSEIGMKGERRRGKGHDGLYQGLSTATKDTYDALHMQALPPR

SEQ ID NO: 62 - protein, 363 aa, Artificial Sequence
  CD70-CAR-1F
MALPVTALLLPLALLLHAARPEVQVVESGGGMVQAGGSLRLSCAASGKRFSFYFMGWYRQAPGKQRELVALITGDGRTNYAGSVEGRFTISRDNAKNTLYLQMNSMKPEDTAVYYCYADAFAGAGRDEYWGQGTQVSVSSTTTPAPRPPTPAPTIASQPLSLRPEACRPAAGGAVHTRGLDFACDIYIWAPLAGTCGVLLLSLVITLYCKRGRKKLLYIFKQPFMRPVQTTQEEDGCSCRFPEEEEGGCELRVKFSRSADAPAYKQGQNQLYNELNLGRREEYDVLDKRRGRDPEMGGKPRRKNPQEGLYNELQKDKMAEAYSEIGMKGERRRGKGHDGLYQGLSTATKDTYDALHMQALPPR

SEQ ID NO: 63 - protein, 362 aa, Artificial Sequence
  CD70-CAR-1G
MALPVTALLLPLALLLHAARPQLQLVESGGGLVQLGGSLTLSCTASGIIFNSDYVGWYRQAPGSDRELVALTSNMRTNYADSVEGRFTISRDNAKNTVYLQMNSLKPEDTAVYYCNVNRMTSYGPRDYWGQGTQVTVSSTTTPAPRPPTPAPTIASQPLSLRPEACRPAAGGAVHTRGLDFACDIYIWAPLAGTCGVLLLSLVITLYCKRGRKKLLYIFKQPFMRPVQTTQEEDGCSCRFPEEEEGGCELRVKFSRSADAPAYKQGQNQLYNELNLGRREEYDVLDKRRGRDPEMGGKPRRKNPQEGLYNELQKDKMAEAYSEIGMKGERRRGKGHDGLYQGLSTATKDTYDALHMQALPPR

SEQ ID NO: 64 - protein, 363 aa, Artificial Sequence
  CD70-CAR-1H
MALPVTALLLPLALLLHAARPEVQLVESGGGMVQAGGSLRLSCAASGKPFSFYFMGWYRQAPGKQRELVALITGDGMTNYADSVEGRFTISRDNAKNTMYLQMNSLKPEDTAVYYCYADVWAGAGRDEYWGQGTRVTVSSTTTPAPRPPTPAPTIASQPLSLRPEACRPAAGGAVHTRGLDFACDIYIWAPLAGTCGVLLLSLVITLYCKRGRKKLLYIFKQPFMRPVQTTQEEDGCSCRFPEEEEGGCELRVKFSRSADAPAYKQGQNQLYNELNLGRREEYDVLDKRRGRDPEMGGKPRRKNPQEGLYNELQKDKMAEAYSEIGMKGERRRGKGHDGLYQGLSTATKDTYDALHMQALPPR

SEQ ID NO: 65 - protein, 361 aa, Artificial Sequence
  CD70-CAR-3H
MALPVTALLLPLALLLHAARPQLQLVESGGGLVQPGGSLRLSCAASGNILRFNAVGWYRQAPGKQRDLVAAMAGARTNYADSVEGRFTISGNNANNTVYLQMNSLKPEDTGVYYCGADRVYGPPYEYGGRGTQVTVLSTTTPAPRPPTPAPTIASQPLSLRPEACRPAAGGAVHTRGLDFACDIYIWAPLAGTCGVLLLSLVITLYCKRGRKKLLYIFKQPFMRPVQTTQEEDGCSCRFPEEEEGGCELRVKFSRSADAPAYKQGQNQLYNELNLGRREEYDVLDKRRGRDPEMGGKPRRKNPQEGLYNELQKDKMAEAYSEIGMKGERRRGKGHDGLYQGLSTATKDTYDALHMQALPPR

SEQ ID NO: 66 - protein, 356 aa, Artificial Sequence
  CD70-CAR-5A
MALPVTALLLPLALLLHAARPEVQLVESGGGLVQAGGSLRLSCAASESIFNNYVMAWYRQPPGKQREAVAQISTDGSAYYQDRVKGRFTISRDNAKNLVNLQMSSLKPEDTAVYYCTAGLQYWGQGTQVTVSSTTTPAPRPPTPAPTIASQPLSLRPEACRPAAGGAVHTRGLDFACDIYIWAPLAGTCGVLLLSLVITLYCKRGRKKLLYIFKQPFMRPVQTTQEEDGCSCRFPEEEEGGCELRVKFSRSADAPAYKQGQNQLYNELNLGRREEYDVLDKRRGRDPEMGGKPRRKNPQEGLYNELQKDKMAEAYSEIGMKGERRRGKGHDGLYQGLSTATKDTYDALHMQALPPR

SEQ ID NO: 67 - protein, 370 aa, Artificial Sequence
  CD70-CAR-5B
MALPVTALLLPLALLLHAARPQVQLVESGGGLVQAGGSLRLSCAASGFTFDDYAIGWFRQAPGKEPEGVSCFRSSDGNIYYSDSVRGRFTISSDNAKNTVYLQMNRLKPEDTAVYYCAAYSVLLRPWVLCEGSYDYWGQGTQVTVSSTTTPAPRPPTPAPTIASQPLSLRPEACRPAAGGAVHTRGLDFACDIYIWAPLAGTCGVLLLSLVITLYCKRGRKKLLYIFKQPFMRPVQTTQEEDGCSCRFPEEEEGGCELRVKFSRSADAPAYKQGQNQLYNELNLGRREEYDVLDKRRGRDPEMGGKPRRKNPQEGLYNELQKDKMAEAYSEIGMKGERRRGKGHDGLYQGLSTATKDTYDALHMQALPPR

SEQ ID NO: 68 - protein, 363 aa, Artificial Sequence
  CD70-CAR-5H
MALPVTALLLPLALLLHAARPEVQLVESGGGMVQAGGSLRLSCAAPGKIFSFYFMGWYRQAPGKQRELVALITGDGRTNYADSVEGRFTISRDNAKNTVYLQMNSLKPEDTAVYYCYADVFARAGRDEYWGQGTQVSVSSTTTPAPRPPTPAPTIASQPLSLRPEACRPAAGGAVHTRGLDFACDIYIWAPLAGTCGVLLLSLVITLYCKRGRKKLLYIFKQPFMRPVQTTQEEDGCSCRFPEEEEGGCELRVKFSRSADAPAYKQGQNQLYNELNLGRREEYDVLDKRRGRDPEMGGKPRRKNPQEGLYNELQKDKMAEAYSEIGMKGERRRGKGHDGLYQGLSTATKDTYDALHMQALPPR

SEQ ID NO: 69 - protein, 369 aa, Artificial Sequence
  CD70-CAR-7D
MALPVTALLLPLALLLHAARPEVQLVESGGGLVQAGGSLRLSCAASGFTFDDYAIGWFRQAPGKEQEGVSCIRRSDGSTWYANSVKGRFTISNDNAKNTVYLQMNSLKPEDTAVYYCAVDRYGQSWHEGRGALDAWGQGTLVTVSSTTTPAPRPPTPAPTIASQPLSLRPEACRPAAGGAVHTRGLDFACDIYIWAPLAGTCGVLLLSLVITLYCKRGRKKLLYIFKQPFMRPVQTTQEEDGCSCRFPEEEEGGCELRVKFSRSADAPAYKQGQNQLYNELNLGRREEYDVLDKRRGRDPEMGGKPRRKNPQEGLYNELQKDKMAEAYSEIGMKGERRRGKGHDGLYQGLSTATKDTYDALHMQALPPR

SEQ ID NO: 70 - protein, 363 aa, Artificial Sequence
  CD70-CAR-H3
MALPVTALLLPLALLLHAARPQVQLVESGGGMVQAGRSLRLSCAASGKPFSFYFMGWYRQAPGKERELVALITGDGMTNYADSVEGRFTISRDNAKNTLYLEMNSLKPEDTAVYYCYADAWAGAVRAEYWGQGTQVSVSSTTTPAPRPPTPAPTIASQPLSLRPEACRPAAGGAVHTRGLDFACDIYIWAPLAGTCGVLLLSLVITLYCKRGRKKLLYIFKQPFMRPVQTTQEEDGCSCRFPEEEEGGCELRVKFSRSADAPAYKQGQNQLYNELNLGRREEYDVLDKRRGRDPEMGGKPRRKNPQEGLYNELQKDKMAEAYSEIGMKGERRRGKGHDGLYQGLSTATKDTYDALHMQALPPR

SEQ ID NO: 71 - protein, 369 aa, Artificial Sequence
  CD70-CAR-L2
MALPVTALLLPLALLLHAARPEVQLVESGGGLVQAGGSLRLSCAASGFTVDDYVIGWFRQAPGKEHEGVSCISSNDGSTWYADSVKGRFTISSDNAKNTMYLQMNSLKPEDTAVYYCAAKYAPYGLEYWEGGMDYWGKGTLVTVSSTTTPAPRPPTPAPTIASQPLSLRPEACRPAAGGAVHTRGLDFACDIYIWAPLAGTCGVLLLSLVITLYCKRGRKKLLYIFKQPFMRPVQTTQEEDGCSCRFPEEEEGGCELRVKFSRSADAPAYKQGQNQLYNELNLGRREEYDVLDKRRGRDPEMGGKPRRKNPQEGLYNELQKDKMAEAYSEIGMKGERRRGKGHDGLYQGLSTATKDTYDALHMQALPPR

SEQ ID NO: 72 - protein, 368 aa, Artificial Sequence
  CD70-CAR-L1
MALPVTALLLPLALLLHAARPEVQVVESGGGLVQAGGSLRLSCAASGRTFSSYAMGWVRQAPGKDQEFVAAINWSDGSTYYADSVKGRFTIARDNAKNTAFLQMNSLKPEDTAVYYCAAGCCGVADAPLNALDAWGQGTLVTVSSTTTPAPRPPTPAPTIASQPLSLRPEACRPAAGGAVHTRGLDFACDIYIWAPLAGTCGVLLLSLVITLYCKRGRKKLLYIFKQPFMRPVQTTQEEDGCSCRFPEEEEGGCELRVKFSRSADAPAYKQGQNQLYNELNLGRREEYDVLDKRRGRDPEMGGKPRRKNPQEGLYNELQKDKMAEAYSEIGMKGERRRGKGHDGLYQGLSTATKDTYDALHMQALPPR

SEQ ID NO: 73 - DNA, 1089 bp, Artificial Sequence
  Nucleic acid sequence of CD70-CAR-1C
atggccttaccagtgaccgccttgctcctgccgctggccttgctgctccacgccgccaggccggaggtgcaggtggtggagtcggggggaggaatggtgcaggctgggcgatctctgagactctcctgtgctgcctctggaaagcccttcagtttctatttcatgggatggtatcgccaggctccaggaaaccagcgcgagttggtcgcccttattaccggtgatggtatgacaaactatgcagactccgtggagggccgattcaccatctccagagacaacgccaagaatacaatgtatctcgaaatgaacagcctgaaacctgaggacacagccgtctattattgctatgcagatgcttgggcgggggccggccgcgaagagtactggggccaggggacccaggtcagcgtctcctcaaccacgacgccagcgccgcgaccaccaacaccggcgcccaccatcgcgtcgcagcccctgtccctgcgcccagaggcgtgccggccagcggcggggggcgcagtgcacacgagggggctggacttcgcctgtgatatctacatctgggcgcccttggccgggacttgtggggtccttctcctgtcactggttatcaccctttactgcaaacggggcagaaagaaactcctgtatatattcaaacaaccatttatgagaccagtacaaactactcaagaggaagatggctgtagctgccgatttccagaagaagaagaaggaggatgtgaactgagagtgaagttcagcaggagcgcagacgcccccgcgtacaagcagggccagaaccagctctataacgagctcaatctaggacgaagagaggagtacgatgttttggacaagagacgtggccgggaccctgagatggggggaaagccgagaaggaagaaccctcaggaaggcctgtacaatgaactgcagaaagataagatggcggaggcctacagtgagattgggatgaaaggcgagcgccggaggggcaaggggcacgatggcctttaccagggtctcagtacagccaccaaggacacctacgacgcccttcacatgcaggccctgccccctcgc

SEQ ID NO: 74 - DNA, 1107 bp, Artificial Sequence
  Nucleic acid sequence of CD70-CAR-1E
atggccttaccagtgaccgccttgctcctgccgctggccttgctgctccacgccgccaggccggaggtgcaggtggtggagtctgggggaggcttggtgcaggctggggggtctctgagactctcctgtgcagcctctggattcgctttcgatgattatgccataggctggttccgccaggccccagggaaggagcaggaaagagtctcatgtatgagtagtagtgatggtagcacatactatgcagactccgtgaagggccgattcaccatctccagtgacaacgccaagaacacggtgtatctgcaaatgaacagcctgaaacctgaggacacggccgtttattactgtgccgcaggggtcaattactatcgcgaggatgggtgcccgggcgcgttggactactggggccaggggacccaggtcaccgtctcctcaaccacgacgccagcgccgcgaccaccaacaccggcgcccaccatcgcgtcgcagcccctgtccctgcgcccagaggcgtgccggccagcggcggggggcgcagtgcacacgagggggctggacttcgcctgtgatatctacatctgggcgcccttggccgggacttgtggggtccttctcctgtcactggttatcaccctttactgcaaacggggcagaaagaaactcctgtatatattcaaacaaccatttatgagaccagtacaaactactcaagaggaagatggctgtagctgccgatttccagaagaagaagaaggaggatgtgaactgagagtgaagttcagcaggagcgcagacgcccccgcgtacaagcagggccagaaccagctctataacgagctcaatctaggacgaagagaggagtacgatgttttggacaagagacgtggccgggaccctgagatggggggaaagccgagaaggaagaaccctcaggaaggcctgtacaatgaactgcagaaagataagatggcggaggcctacagtgagattgggatgaaaggcgagcgccggaggggcaaggggcacgatggcctttaccagggtctcagtacagccaccaaggacacctacgacgcccttcacatgcaggccctgccccctcgc

SEQ ID NO: 75 - DNA, 1089 bp, Artificial Sequence
  Nucleic acid sequence of CD70-CAR-1F
atggccttaccagtgaccgccttgctcctgccgctggccttgctgctccacgccgccaggccggaggtgcaggtggtggagtcggggggaggaatggtgcaggctgggggatctctgaggctctcctgtgcagcctctggaaagcgcttcagtttctattttatgggatggtaccgccaggctccaggaaagcagcgcgagttggtcgcccttattactggtgatggcaggacaaactatgcagggtccgtggagggccgattcaccatctccagagacaacgccaagaacacgctatatctgcaaatgaacagcatgaaacctgaggacacagccgtctattattgctatgcagatgcattcgcgggggccggccgcgatgagtactggggccaggggacccaggtcagcgtctcctcaaccacgacgccagcgccgcgaccaccaacaccggcgcccaccatcgcgtcgcagcccctgtccctgcgcccagaggcgtgccggccagcggcggggggcgcagtgcacacgagggggctggacttcgcctgtgatatctacatctgggcgcccttggccgggacttgtggggtccttctcctgtcactggttatcaccctttactgcaaacggggcagaaagaaactcctgtatatattcaaacaaccatttatgagaccagtacaaactactcaagaggaagatggctgtagctgccgatttccagaagaagaagaaggaggatgtgaactgagagtgaagttcagcaggagcgcagacgcccccgcgtacaagcagggccagaaccagctctataacgagctcaatctaggacgaagagaggagtacgatgttttggacaagagacgtggccgggaccctgagatggggggaaagccgagaaggaagaaccctcaggaaggcctgtacaatgaactgcagaaagataagatggcggaggcctacagtgagattgggatgaaaggcgagcgccggaggggcaaggggcacgatggcctttaccagggtctcagtacagccaccaaggacacctacgacgcccttcacatgcaggccctgccccctcgc

SEQ ID NO: 76 - DNA, 1086 bp, Artificial Sequence
  Nucleic acid sequence of CD70-CAR-1G
atggccttaccagtgaccgccttgctcctgccgctggccttgctgctccacgccgccaggccgcagttgcagctcgtggagtccgggggaggcttggtgcaacttggggggtctctgacgctctcctgtacagcctctgggattatcttcaatagcgattacgtgggctggtaccgccaggctccagggtcggatcgcgagttggtcgcacttactagtaatatgaggacaaactatgcagactccgtggagggccgattcaccatctccagagacaacgccaagaatacggtgtatctgcaaatgaacagcctgaaacctgaggacacggccgtctattattgtaatgtaaatagaatgacctcctatgggcctcgggactactggggccaggggacccaggtcaccgtctcctccaccacgacgccagcgccgcgaccaccaacaccggcgcccaccatcgcgtcgcagcccctgtccctgcgcccagaggcgtgccggccagcggcggggggcgcagtgcacacgagggggctggacttcgcctgtgatatctacatctgggcgcccttggccgggacttgtggggtccttctcctgtcactggttatcaccctttactgcaaacggggcagaaagaaactcctgtatatattcaaacaaccatttatgagaccagtacaaactactcaagaggaagatggctgtagctgccgatttccagaagaagaagaaggaggatgtgaactgagagtgaagttcagcaggagcgcagacgcccccgcgtacaagcagggccagaaccagctctataacgagctcaatctaggacgaagagaggagtacgatgttttggacaagagacgtggccgggaccctgagatggggggaaagccgagaaggaagaaccctcaggaaggcctgtacaatgaactgcagaaagataagatggcggaggcctacagtgagattgggatgaaaggcgagcgccggaggggcaaggggcacgatggcctttaccagggtctcagtacagccaccaaggacacctacgacgcccttcacatgcaggccctgccccctcgc

SEQ ID NO: 77 - DNA, 1089 bp, Artificial Sequence
  Nucleic acid sequence of CD70-CAR-1H
atggccttaccagtgaccgccttgctcctgccgctggccttgctgctccacgccgccaggccggaggtgcagctggtggagtctggtggaggaatggtgcaggctgggggatctctgagactctcctgtgctgcctctggaaagcccttcagtttctatttcatgggatggtaccgccaggctccaggaaagcagcgcgagttggtcgcccttattaccggtgatggtatgacaaactatgcagactccgtggagggccgattcaccatctccagagacaacgccaagaacacaatgtatctgcaaatgaacagcctgaaacctgaggacacagccgtctattattgctatgcagatgtatgggcgggggccggccgcgatgagtactggggccaggggacccgggtcaccgtctcctcaaccacgacgccagcgccgcgaccaccaacaccggcgcccaccatcgcgtcgcagcccctgtccctgcgcccagaggcgtgccggccagcggcggggggcgcagtgcacacgagggggctggacttcgcctgtgatatctacatctgggcgcccttggccgggacttgtggggtccttctcctgtcactggttatcaccctttactgcaaacggggcagaaagaaactcctgtatatattcaaacaaccatttatgagaccagtacaaactactcaagaggaagatggctgtagctgccgatttccagaagaagaagaaggaggatgtgaactgagagtgaagttcagcaggagcgcagacgcccccgcgtacaagcagggccagaaccagctctataacgagctcaatctaggacgaagagaggagtacgatgttttggacaagagacgtggccgggaccctgagatggggggaaagccgagaaggaagaaccctcaggaaggcctgtacaatgaactgcagaaagataagatggcggaggcctacagtgagattgggatgaaaggcgagcgccggaggggcaaggggcacgatggcctttaccagggtctcagtacagccaccaaggacacctacgacgcccttcacatgcaggccctgccccctcgc

SEQ ID NO: 78 - DNA, 1083 bp, Artificial Sequence
  Nucleic acid sequence of CD70-CAR-3H
atggccttaccagtgaccgccttgctcctgccgctggccttgctgctccacgccgccaggccgcagttgcagctcgtggagtcgggtggaggcttggtgcagcctggggggtctctgagactctcctgtgcagcctctggaaacatcctcagattcaatgccgtgggctggtaccgccaggctccagggaagcagcgcgacttggtcgcggctatggctggtgcacggacaaactatgcagactccgtggagggccgattcaccatctccggaaacaacgccaacaacacggtttatctgcaaatgaacagcctgaaacctgaagacacaggcgtctactactgtggtgctgaccgcgtatatggtccgccgtatgaatatgggggccgggggacccaggtcaccgtcttgtcaaccacgacgccagcgccgcgaccaccaacaccggcgcccaccatcgcgtcgcagcccctgtccctgcgcccagaggcgtgccggccagcggcggggggcgcagtgcacacgagggggctggacttcgcctgtgatatctacatctgggcgcccttggccgggacttgtggggtccttctcctgtcactggttatcaccctttactgcaaacggggcagaaagaaactcctgtatatattcaaacaaccatttatgagaccagtacaaactactcaagaggaagatggctgtagctgccgatttccagaagaagaagaaggaggatgtgaactgagagtgaagttcagcaggagcgcagacgcccccgcgtacaagcagggccagaaccagctctataacgagctcaatctaggacgaagagaggagtacgatgttttggacaagagacgtggccgggaccctgagatggggggaaagccgagaaggaagaaccctcaggaaggcctgtacaatgaactgcagaaagataagatggcggaggcctacagtgagattgggatgaaaggcgagcgccggaggggcaaggggcacgatggcctttaccagggtctcagtacagccaccaaggacacctacgacgcccttcacatgcaggccctgccccctcgc

SEQ ID NO: 79 - DNA, 1068 bp, Artificial Sequence
  Nucleic acid sequence of CD70-CAR-5A
atggccttaccagtgaccgccttgctcctgccgctggccttgctgctccacgccgccaggccggaggtgcagctggtggagtcggggggaggcttggtgcaggctggggggtctctgaggctctcctgtgcagcctctgaaagcatcttcaataattatgtcatggcctggtaccgccagcctccagggaagcagcgcgaggcggtcgcacaaattagtactgatggtagtgcgtactatcaggaccgagtgaagggccgattcactatctccagagacaacgccaagaacttggtgaatctgcaaatgagcagcctgaaacctgaggacacagccgtctattactgtactgcaggtctccagtactggggccaggggacccaggtcaccgtctcctcaaccacgacgccagcgccgcgaccaccaacaccggcgcccaccatcgcgtcgcagcccctgtccctgcgcccagaggcgtgccggccagcggcggggggcgcagtgcacacgagggggctggacttcgcctgtgatatctacatctgggcgcccttggccgggacttgtggggtccttctcctgtcactggttatcaccctttactgcaaacggggcagaaagaaactcctgtatatattcaaacaaccatttatgagaccagtacaaactactcaagaggaagatggctgtagctgccgatttccagaagaagaagaaggaggatgtgaactgagagtgaagttcagcaggagcgcagacgcccccgcgtacaagcagggccagaaccagctctataacgagctcaatctaggacgaagagaggagtacgatgttttggacaagagacgtggccgggaccctgagatggggggaaagccgagaaggaagaaccctcaggaaggcctgtacaatgaactgcagaaagataagatggcggaggcctacagtgagattgggatgaaaggcgagcgccggaggggcaaggggcacgatggcctttaccagggtctcagtacagccaccaaggacacctacgacgcccttcacatgcaggccctgccccctcgc

SEQ ID NO: 80 - DNA, 1110 bp, Artificial Sequence
  Nucleic acid sequence of CD70-CAR-5B
atggccttaccagtgaccgccttgctcctgccgctggccttgctgctccacgccgccaggccgcaggtgcagctcgtggagtctggaggaggcttggtgcaggctggggggtctctgagactctcctgtgcagcctctggattcactttcgatgattatgccataggctggttccgccaggccccagggaaggagcctgagggggtctcatgtttcaggagtagtgatggtaacatatactattcagactccgtgaggggccgattcaccatctccagtgacaacgccaagaacacggtgtatctgcaaatgaacagactgaaacctgaggacacggccgtttactactgtgcagcctatagcgtactgctcaggccctgggtgttatgtgaaggctcatatgactactggggccaggggacccaggtcaccgtctcctcaaccacgacgccagcgccgcgaccaccaacaccggcgcccaccatcgcgtcgcagcccctgtccctgcgcccagaggcgtgccggccagcggcggggggcgcagtgcacacgagggggctggacttcgcctgtgatatctacatctgggcgcccttggccgggacttgtggggtccttctcctgtcactggttatcaccctttactgcaaacggggcagaaagaaactcctgtatatattcaaacaaccatttatgagaccagtacaaactactcaagaggaagatggctgtagctgccgatttccagaagaagaagaaggaggatgtgaactgagagtgaagttcagcaggagcgcagacgcccccgcgtacaagcagggccagaaccagctctataacgagctcaatctaggacgaagagaggagtacgatgttttggacaagagacgtggccgggaccctgagatggggggaaagccgagaaggaagaaccctcaggaaggcctgtacaatgaactgcagaaagataagatggcggaggcctacagtgagattgggatgaaaggcgagcgccggaggggcaaggggcacgatggcctttaccagggtctcagtacagccaccaaggacacctacgacgcccttcacatgcaggccctgccccctcgc

SEQ ID NO: 81 - DNA, 1089 bp, Artificial Sequence
  Nucleic acid sequence of CD70-CAR-5H
atggccttaccagtgaccgccttgctcctgccgctggccttgctgctccacgccgccaggccggaggtgcagctggtggagtcagggggaggtatggtgcaggctgggggatctctgagactctcctgtgcagcccctggaaagatcttcagtttctatttcatgggatggtaccgccaggctccaggaaagcagcgcgagttggtcgcccttattaccggtgatggtaggacaaactatgcagactccgtggagggccgattcaccatctccagagacaacgccaagaacacggtgtatctgcaaatgaacagcctgaaacctgaggacacagccgtctattattgctatgcagatgtatttgcgagggccggccgcgatgagtactggggccaggggacccaggtcagcgtctcctcaaccacgacgccagcgccgcgaccaccaacaccggcgcccaccatcgcgtcgcagcccctgtccctgcgcccagaggcgtgccggccagcggcggggggcgcagtgcacacgagggggctggacttcgcctgtgatatctacatctgggcgcccttggccgggacttgtggggtccttctcctgtcactggttatcaccctttactgcaaacggggcagaaagaaactcctgtatatattcaaacaaccatttatgagaccagtacaaactactcaagaggaagatggctgtagctgccgatttccagaagaagaagaaggaggatgtgaactgagagtgaagttcagcaggagcgcagacgcccccgcgtacaagcagggccagaaccagctctataacgagctcaatctaggacgaagagaggagtacgatgttttggacaagagacgtggccgggaccctgagatggggggaaagccgagaaggaagaaccctcaggaaggcctgtacaatgaactgcagaaagataagatggcggaggcctacagtgagattgggatgaaaggcgagcgccggaggggcaaggggcacgatggcctttaccagggtctcagtacagccaccaaggacacctacgacgcccttcacatgcaggccctgccccctcgc

SEQ ID NO: 82 - DNA, 1107 bp, Artificial Sequence
  Nucleic acid sequence of CD70-CAR-7D
atggccttaccagtgaccgccttgctcctgccgctggccttgctgctccacgccgccaggccggaggtgcagctggtggagtctgggggaggcttggtgcaggctggggggtctctgagactctcctgtgcagcctctggattcactttcgatgattatgccataggctggttccgccaggccccagggaaggagcaagagggggtctcatgtattagacgtagtgatggtagcacatggtatgcaaactccgtgaagggccgattcaccatctccaatgacaacgccaagaacacggtgtatctgcaaatgaacagcctgaaacctgaggacacggccgtttattactgcgcagtagatcgttacggtcagagttggcacgagggccgcggcgctttggacgcatggggccaggggaccctggtcactgtctcctcaaccacgacgccagcgccgcgaccaccaacaccggcgcccaccatcgcgtcgcagcccctgtccctgcgcccagaggcgtgccggccagcggcggggggcgcagtgcacacgagggggctggacttcgcctgtgatatctacatctgggcgcccttggccgggacttgtggggtccttctcctgtcactggttatcaccctttactgcaaacggggcagaaagaaactcctgtatatattcaaacaaccatttatgagaccagtacaaactactcaagaggaagatggctgtagctgccgatttccagaagaagaagaaggaggatgtgaactgagagtgaagttcagcaggagcgcagacgcccccgcgtacaagcagggccagaaccagctctataacgagctcaatctaggacgaagagaggagtacgatgttttggacaagagacgtggccgggaccctgagatggggggaaagccgagaaggaagaaccctcaggaaggcctgtacaatgaactgcagaaagataagatggcggaggcctacagtgagattgggatgaaaggcgagcgccggaggggcaaggggcacgatggcctttaccagggtctcagtacagccaccaaggacacctacgacgcccttcacatgcaggccctgccccctcgc

SEQ ID NO: 83 - DNA, 1089 bp, Artificial Sequence
  Nucleic acid sequence of CD70-CAR-H3
atggccttaccagtgaccgccttgctcctgccgctggccttgctgctccacgccgccaggccgcaggtgcagctcgtggagtctgggggaggaatggtgcaggctgggcgatctctgagactctcctgtgctgcctctggaaagcccttcagtttctatttcatgggatggtatcgccaggctccaggaaaggagcgcgagttggtcgcccttattaccggtgatggtatgacaaactatgcagactccgtggagggccgattcaccatctccagagacaacgccaagaatacattgtatctcgaaatgaacagcctgaaacctgaggacacagccgtctattattgctatgcagatgcttgggcgggggccgttcgcgccgagtactggggccaggggacccaggtcagcgtctcctcaaccacgacgccagcgccgcgaccaccaacaccggcgcccaccatcgcgtcgcagcccctgtccctgcgcccagaggcgtgccggccagcggcggggggcgcagtgcacacgagggggctggacttcgcctgtgatatctacatctgggcgcccttggccgggacttgtggggtccttctcctgtcactggttatcaccctttactgcaaacggggcagaaagaaactcctgtatatattcaaacaaccatttatgagaccagtacaaactactcaagaggaagatggctgtagctgccgatttccagaagaagaagaaggaggatgtgaactgagagtgaagttcagcaggagcgcagacgcccccgcgtacaagcagggccagaaccagctctataacgagctcaatctaggacgaagagaggagtacgatgttttggacaagagacgtggccgggaccctgagatggggggaaagccgagaaggaagaaccctcaggaaggcctgtacaatgaactgcagaaagataagatggcggaggcctacagtgagattgggatgaaaggcgagcgccggaggggcaaggggcacgatggcctttaccagggtctcagtacagccaccaaggacacctacgacgcccttcacatgcaggccctgccccctcgc

SEQ ID NO: 84 - DNA, 1107 bp, Artificial Sequence
  Nucleic acid sequence of CD70-CAR-L2
atggccttaccagtgaccgccttgctcctgccgctggccttgctgctccacgccgccaggccggaggtgcagctggtggagtccgggggaggcttggtgcaggctggggggtctctgagactctcctgtgcagcctctggattcactgtcgatgattatgtcataggctggttccgccaggccccagggaaggagcatgagggggtctcatgtattagtagtaatgatggtagtacatggtatgcagactccgtgaagggccgattcaccatctccagtgacaacgccaagaacacgatgtatctgcaaatgaacagcctgaaacctgaggacacggccgtttattactgtgcagctaaatacgcaccctacgggttggagtactgggagggaggcatggactactggggcaaagggaccctggtcaccgtctcctcaaccacgacgccagcgccgcgaccaccaacaccggcgcccaccatcgcgtcgcagcccctgtccctgcgcccagaggcgtgccggccagcggcggggggcgcagtgcacacgagggggctggacttcgcctgtgatatctacatctgggcgcccttggccgggacttgtggggtccttctcctgtcactggttatcaccctttactgcaaacggggcagaaagaaactcctgtatatattcaaacaaccatttatgagaccagtacaaactactcaagaggaagatggctgtagctgccgatttccagaagaagaagaaggaggatgtgaactgagagtgaagttcagcaggagcgcagacgcccccgcgtacaagcagggccagaaccagctctataacgagctcaatctaggacgaagagaggagtacgatgttttggacaagagacgtggccgggaccctgagatggggggaaagccgagaaggaagaaccctcaggaaggcctgtacaatgaactgcagaaagataagatggcggaggcctacagtgagattgggatgaaaggcgagcgccggaggggcaaggggcacgatggcctttaccagggtctcagtacagccaccaaggacacctacgacgcccttcacatgcaggccctgccccctcgc

SEQ ID NO: 85 - DNA, 1104 bp, Artificial Sequence
  Nucleic acid sequence of CD70-CAR-L1
atggccttaccagtgaccgccttgctcctgccgctggccttgctgctccacgccgccaggccggaggtgcaggtggtggagtctgggggaggattggtgcaggctgggggctctctgagactctcctgtgcagcctctggacgcaccttcagttcatatgccatgggctgggtccgccaggctccagggaaggaccaagagtttgtagcggctattaactggagtgatggtagcacatactatgcagactccgtgaagggccgattcaccatcgccagagacaacgccaagaacacggcgtttctgcaaatgaacagcctgaaacctgaggacacggccgtgtattactgtgcagcagggtgttgcggagtagctgatgcccccctcaatgctttggacgcatggggccaggggaccctggtcactgtctcctcaaccacgacgccagcgccgcgaccaccaacaccggcgcccaccatcgcgtcgcagcccctgtccctgcgcccagaggcgtgccggccagcggcggggggcgcagtgcacacgagggggctggacttcgcctgtgatatctacatctgggcgcccttggccgggacttgtggggtccttctcctgtcactggttatcaccctttactgcaaacggggcagaaagaaactcctgtatatattcaaacaaccatttatgagaccagtacaaactactcaagaggaagatggctgtagctgccgatttccagaagaagaagaaggaggatgtgaactgagagtgaagttcagcaggagcgcagacgcccccgcgtacaagcagggccagaaccagctctataacgagctcaatctaggacgaagagaggagtacgatgttttggacaagagacgtggccgggaccctgagatggggggaaagccgagaaggaagaaccctcaggaaggcctgtacaatgaactgcagaaagataagatggcggaggcctacagtgagattgggatgaaaggcgagcgccggaggggcaaggggcacgatggcctttaccagggtctcagtacagccaccaaggacacctacgacgcccttcacatgcaggccctgccccctcgc

SEQ ID NO: 86 - DNA, 21 bp, Artificial Sequence
  Lenti-For
tcaagcctcagacagtggttc

SEQ ID NO: 87 - DNA, 24 bp, Artificial Sequence
  Lenti-Rev
cctcataaagagacagcaaccagg

SEQ ID NO: 88 - DNA, 63 bp, Artificial Sequence
  Signal peptide of CD8α
atggccttaccagtgaccgccttgctcctgccgctggccttgctgctccacgccgccaggccg

SEQ ID NO: 89 - DNA, 135 bp, Artificial Sequence
  Hinge region of CD8α
accacgacgccagcgccgcgaccaccaacaccggcgcccaccatcgcgtcgcagcccctgtccctgcgcccagaggcgtgccggccagcggcggggggcgcagtgcacacgagggggctggacttcgcctgtgat

SEQ ID NO: 90 - DNA, 75 bp, Artificial Sequence
  Transmembrane domain of CD8α
atctacatctgggcgcccttggccgggacttgtggggtccttctcctgtcactggttatcaccctttactgcaaa

SEQ ID NO: 91 - DNA, 120 bp, Artificial Sequence
  Co-stimulatory signaling domain of 4-1BB
cggggcagaaagaaactcctgtatatattcaaacaaccatttatgagaccagtacaaactactcaagaggaagatggctgtagctgccgatttccagaagaagaagaaggaggatgtgaa

SEQ ID NO: 92 - DNA, 339 bp, Artificial Sequence
  Intracellular signaling domain of CD3ζ
ctgagagtgaagttcagcaggagcgcagacgcccccgcgtaccagcagggccagaaccagctctataacgagctcaatctaggacgaagagaggagtacgatgttttggacaagagacgtggccgggaccctgagatggggggaaagccgagaaggaagaaccctcaggaaggcctgtacaatgaactgcagaaagataagatggcggaggcctacagtgagattgggatgaaaggcgagcgccggaggggcaaggggcacgatggcctttaccagggtctcagtacagccaccaaggacacctacgacgcccttcacatgcaggccctgccccctcgc

SEQ ID NO: 93 - DNA, 1518 bp, Artificial Sequence
  Nucleic acid sequence of CD70-CAR-03
atggccttaccagtgaccgccttgctcctgccgctggccttgctgctccacgccgccaggccgggcggcagcgactacaaagacgatgacgacaagggtggctcccaggcagtggtgacccaggagccttccctgacagtgtctccaggagggacggtcacgctcacctgcggcctcaaatctgggtctgtcacttccgataacttccccacttggtaccagcagacaccaggccaggctccccgattgcttatctacaacacaaacacccgtcactctggcgtccccgaccgcttctccggatccatcctgggcaacaaagccgccctcaccatcacgggggcccaggccgacgacgaggccgaatatttctgtgctctgttcataagtaatcctagtgttgagttcggcggagggacccaactgaccgtcctaggtggtggcggtggctcgggcggtggtgggtcgggtggcggcggatctgaggtgcagctcgtggagtctgggggaggcttggtgcagcctggggggtctctgagactctcctgtgcagcctctggattcaccttcagtgtctactacatgaactgggtccgccaggctccagggaaggggctcgagtgggtctcagatattaataatgaaggtggtactacatactatgcagactccgtgaagggccgattcaccatctccagagacaactctaagaacagcctgtatctgcaaatgaacagcctgcgcgccgaggacacggccgtgtactactgcgcgagagatgccggatatagcaaccatgtacccatctttgattcttggggccaggggaccctggtcactgtctcctcaaccacgacgccagcgccgcgaccaccaacaccggcgcccaccatcgcgtcgcagcccctgtccctgcgcccagaggcgtgccggccagcggcggggggcgcagtgcacacgagggggctggacttcgcctgtgatatctacatctgggcgcccttggccgggacttgtggggtccttctcctgtcactggttatcaccctttactgcaaacggggcagaaagaaactcctgtatatattcaaacaaccatttatgagaccagtacaaactactcaagaggaagatggctgtagctgccgatttccagaagaagaagaaggaggatgtgaactgagagtgaagttcagcaggagcgcagacgcccccgcgtaccagcagggccagaaccagctctataacgagctcaatctaggacgaagagaggagtacgatgttttggacaagagacgtggccgggaccctgagatggggggaaagccgagaaggaagaaccctcaggaaggcctgtacaatgaactgcagaaagataagatggcggaggcctacagtgagattgggatgaaaggcgagcgccggaggggcaaggggcacgatggcctttaccagggtctcagtacagccaccaaggacacctacgacgcccttcacatgcaggccctgccccctcgc

SEQ ID NO: 94 - protein, 232 aa, Artificial Sequence
  Human Fc sequence
EPKSADKTHTCPPCPAPELLGGPSVFLFPPKPKDTLMISRTPEVTCVVVDVSHEDPEVKFNWYVDGVEVHNAKTKPREEQYNSTYRVVSVLTVLHQDWLNGKEYKCKVSNKALPAPIEKTISKAKGQPREPQVYTLPPSREEMTKNQVSLTCLVKGFYPSDIAVEWESNGQPENNYKTTPPVLDSDGSFFLYSKLTVDKSRWQQGNVFSCSVMHEALHNHYTQKSLSLSPGK